European Patent Application EP 4 198 512 A1, published June 21, 2023. Title: composition for diagnosing or detecting colorectal cancer for predicting drug responsiveness, composition for preventing or treating colorectal cancer. Applicant: Korea University Research and Business Foundation KOREA INSTITUTE OF SCIENCE AND TECHNOLOGY. The sequence listing filed with the application follows.

SEQUENCE LISTING (2 sequences)

SEQ ID NO: 1 - protein, 8 aa, Artificial Sequence
  Artificial peptide
GFLGGKGG

SEQ ID NO: 2 - protein, 5 aa, Artificial Sequence
  Artificial peptide
CGFLG